European Patent Application EP 4 206 222 A1, published July 5, 2023. Title: SIGNAL PEPTIDE FOR REDUCING END HETEROGENEITY OF HETEROLOGOUS POLYPEPTIDE. Applicant: Jiangsu Hengrui Pharmaceuticals Co., Ltd. Shanghai Hengrui Pharmaceutical Co., Ltd. The sequence listing filed with the application follows.

SEQUENCE LISTING (172 sequences)

SEQ ID NO: 1 - protein, 261 aa, Homo sapiens
  PEPTIDE: Claudin18.2 protein
MAVTACQGLGFVVSLIGIAGIIAATCMDQWSTQDLYNNPVTAVFNYQGLWRSCVRESSGFTECRGYFTLLGLPAMLQAVRALMIVGIVLGAIGLLVSIFALKCIRIGSMEDSAKANMTLTSGIMFIVSGLCAIAGVSVFANMLVTNFWMSTANMYTGMGGMVQTVQTRYTFGAALFVGWVAGGLTLIGGVMMCIACRGLAPEETNYKAVSYHASGHSVAYKPGGFKASTGFGSNTKNKKIYDGGARTEDEVQSYPSKHDYV

SEQ ID NO: 2 - DNA, 3350 bp, Homo sapiens
  gene: Claudin18.2
agaattgcgctgtccacttgtcgtgtggctctgtgtcgacactgtgcgccaccatggccgtgactgcctgtcagggcttggggttcgtggtttcactgattgggattgcgggcatcattgctgccacctgcatggaccagtggagcacccaagacttgtacaacaaccccgtaacagctgttttcaactaccaggggctgtggcgctcctgtgtccgagagagctctggcttcaccgagtgccggggctacttcaccctgctggggctgccagccatgctgcaggcagtgcgagccctgatgatcgtaggcatcgtcctgggtgccattggcctcctggtatccatctttgccctgaaatgcatccgcattggcagcatggaggactctgccaaagccaacatgacactgacctccgggatcatgttcattgtctcaggtctttgtgcaattgctggagtgtctgtgtttgccaacatgctggtgactaacttctggatgtccacagctaacatgtacaccggcatgggtgggatggtgcagactgttcagaccaggtacacatttggtgcggctctgttcgtgggctgggtcgctggaggcctcacactaattgggggtgtgatgatgtgcatcgcctgccggggcctggcaccagaagaaaccaactacaaagccgtttcttatcatgcctcaggccacagtgttgcctacaagcctggaggcttcaaggccagcactggctttgggtccaacaccaaaaacaagaagatatacgatggaggtgcccgcacagaggacgaggtacaatcttatccttccaagcacgactatgtgtaatgctctaagacctctcagcacgggcggaagaaactcccggagagctcacccaaaaaacaaggagatcccatctagatttcttcttgcttttgactcacagctggaagttagaaaagcctcgatttcatctttggagaggccaaatggtcttagcctcagtctctgtctctaaatattccaccataaaacagctgagttatttatgaattagaggctatagctcacattttcaatcctctatttctttttttaaatataactttctactctgatgagagaatgtggttttaatctctctctcacattttgatgatttagacagactccccctcttcctcctagtcaataaacccattgatgatctatttcccagcttatccccaagaaaacttttgaaaggaaagagtagacccaaagatgttattttctgctgtttgaattttgtctccccacccccaacttggctagtaataaacacttactgaagaagaagcaataagagaaagatatttgtaatctctccagcccatgatctcggttttcttacactgtgatcttaaaagttaccaaaccaaagtcattttcagtttgaggcaaccaaacctttctactgctgttgacatcttcttattacagcaacaccattctaggagtttcctgagctctccactggagtcctctttctgtcgcgggtcagaaattgtccctagatgaatgagaaaattattttttttaatttaagtcctaaatatagttaaaataaataatgttttagtaaaatgatacactatctctgtgaaatagcctcacccctacatgtggatagaaggaaatgaaaaaataattgctttgacattgtctatatggtactttgtaaagtcatgcttaagtacaaattccatgaaaagctcactgatcctaattctttccctttgaggtctctatggctctgattgtacatgatagtaagtgtaagccatgtaaaaagtaaataatgtctgggcacagtggctcacgcctgtaatcctagcactttgggaggctgaggaggaaggatcacttgagcccagaagttcgagactagcctgggcaacatggagaagccctgtctctacaaaatacagagagaaaaaatcagccagtcatggtggcctacacctgtagtcccagcattccgggaggctgaggtgggaggatcacttgagcccagggaggttggggctgcagtgagccatgatcacaccactgcactccagccaggtgacatagcgagatcctgtctaaaaaaataaaaaataaataatggaacacagcaagtcctaggaagtaggttaaaactaattctttaaaaaaaaaaaaaagttgagcctgaattaaatgtaatgtttccaagtgacaggtatccacatttgcatggttacaagccactgccagttagcagtagcactttcctggcactgtggtcggttttgttttgttttgctttgtttagagacggggtctcactttccaggctggcctcaaactcctgcactcaagcaattcttctaccctggcctcccaagtagctggaattacaggtgtgcgccatcacaactagctggtggtcagttttgttactctgagagctgttcacttctctgaattcacctagagtggttggaccatcagatgtttgggcaaaactgaaagctctttgcaaccacacaccttccctgagcttacatcactgcccttttgagcagaaagtctaaattccttccaagacagtagaattccatcccagtaccaaagccagataggccccctaggaaactgaggtaagagcagtctctaaaaactacccacagcagcattggtgcaggggaacttggccattaggttattatttgagaggaaagtcctcacatcaatagtacatatgaaagtgacctccaaggggattggtgaatactcataaggatcttcaggctgaacagactatgtctggggaaagaacggattatgccccattaaataacaagttgtgttcaagagtcagagcagtgagctcagaggcccttctcactgagacagcaacatttaaaccaaaccagaggaagtatttgtggaactcactgcctcagtttgggtaaaggatgagcagacaagtcaactaaagaaaaaagaaaagcaaggaggagggttgagcaatctagagcatggagtttgttaagtgctctctggatttgagttgaagagcatccatttgagttgaaggccacagggcacaatgagctctcccttctaccaccagaaagtccctggtcaggtctcaggtagtgcggtgtggctcagctgggtttttaattagcgcattctctatccaacatttaattgtttgaaagcctccatatagttagattgtgctttgtaattttgttgttgttgctctatcttattgtatatgcattgagtattaacctgaatgttttgttacttaaatattaaaaacactgttatcctacagtt

SEQ ID NO: 3 - protein, 120 aa, Mus musculus
  DOMAIN: Heavy chain variable region of mAb1901 murine antibody
EVQLMESGGGLVKPGGSLKLSCAASGFTFSDYGIHWVRQAPEMGLEWIAYISRGSSTIYYADTVKGRFTMSRDNAKNTLFLQMTSLRSEDTAMYYCARGGYDTRNAMDYWGQGTSVTVSS

SEQ ID NO: 4 - protein, 113 aa, Mus musculus
  DOMAIN: Light chain variable region of mAb1901 murine antibody
DIVMTQSPSSLSVSAGEKVTMSCKSSQSLLNSGNQKNYLAWYQQKPGQPPKLLIYGASTRASGVPDRFTGSGSGTDFTLTISSVQAEDLAIYHCQNDLYYPLTFGAGTKLELK

SEQ ID NO: 5 - protein, 118 aa, Mus musculus
  DOMAIN: Heavy chain variable region of mAb1902 murine antibody
EVQLQESGAELVKPGASVKLSCKASGYIFTSYWMHWVKQRPGQGLEWIGMIHPNSGSTNYNEKFKGKATLTLDKSSSTAYMQLSSLPSEDSAVYYCARLKTGNSFDYWGQGTTLTVSS

SEQ ID NO: 6 - protein, 113 aa, Mus musculus
  DOMAIN: Light chain variable region of mAb1902 murine antibody
DIVLTQSPSSLTVTAGEKVTMSCKSSQSLLNSGNQKNYLTWYQQKPGQPPKLLIYWASTRESGVPDRFTGSGSGTDFTLTISSVQAEDLAIYYCQNAYTYPFTFGSGTKLEIK

SEQ ID NO: 7 - protein, 330 aa, Homo sapiens [sequence omitted]

SEQ ID NO: 8 - protein, 107 aa, Homo sapiens [sequence omitted]

SEQ ID NO: 9 - protein, 5 aa, Artificial Sequence
  DOMAIN: mAb1901 HCDR1
DYGIH

SEQ ID NO: 10 - protein, 17 aa, Artificial Sequence
  DOMAIN: mAb1901 HCDR2
YISRGSSTIYYADTVKG

SEQ ID NO: 11 - protein, 11 aa, Artificial Sequence
  DOMAIN: mAb1901 HCDR3
GGYDTRNAMDY

SEQ ID NO: 12 - protein, 17 aa, Artificial Sequence
  DOMAIN: mAb1901 LCDR1
KSSQSLLNSGNQKNYLA

SEQ ID NO: 13 - protein, 7 aa, Artificial Sequence
  DOMAIN: mAb1901 LCDR2
GASTRAS

SEQ ID NO: 14 - protein, 9 aa, Artificial Sequence
  DOMAIN: mAb1901 LCDR3
QNDLYYPLT

SEQ ID NO: 15 - protein, 5 aa, Artificial Sequence
  DOMAIN: mAb1902 HCDR1
SYWMH

SEQ ID NO: 16 - protein, 18 aa, Artificial Sequence
  DOMAIN: mAb1902 HCDR2
MIHPNSGSTNYNEKFKGR

SEQ ID NO: 17 - protein, 9 aa, Artificial Sequence
  DOMAIN: mAb1902 HCDR3
LKTGNSFDY

SEQ ID NO: 18 - protein, 17 aa, Artificial Sequence
  DOMAIN: mAb1902 LCDR1
KSSQSLLNSGNQKNYLT

SEQ ID NO: 19 - protein, 7 aa, Artificial Sequence
  DOMAIN: mAb1902 LCDR2
WASTRES

SEQ ID NO: 20 - protein, 9 aa, Artificial Sequence
  DOMAIN: mAb1902 LCDR3
QNAYTYPFT

SEQ ID NO: 21 - protein, 113 aa, Artificial Sequence
  DOMAIN: VL1
DIVMTQSPDSLAVSLGERATINCKSSQSLLNSGNQKNYLAWYQQKPGQPPKLLIYGASTRASGVPDRFSGSGSGTDFTLTISSLQAEDVAVYYCQNDLYYPLTFGQGTKLEIK

SEQ ID NO: 22 - protein, 113 aa, Artificial Sequence
  DOMAIN: VL2
DIVMTQSPDSLAVSLGERATISCKSSQSLLNSGNQKNYLAWYQQKPGQPPKLLIYGASTRASGVPDRFSGSGSGTDFTLTISSLQAEDVAVYYCQNDLYYPLTFGQGTKLEIK

SEQ ID NO: 23 - protein, 113 aa, Artificial Sequence
  DOMAIN: VL3
DIVMTQSPDSLAVSLGERATISCKSSQSLLNSGNQKNYLAWYQQKPGQPPKLLIYGASTRASGVPDRFSGSGSGTDFTLTISSLQAEDVAIYHCQNDLYYPLTFGQGTKLEIK

SEQ ID NO: 24 - protein, 120 aa, Artificial Sequence
  DOMAIN: VH1
EVQLVESGGGLVQPGGSLRLSCAASGFTFSDYGIHWVRQAPGKGLEWVAYISRGSSTIYYADTVKGRFTISRDNAKNSLYLQMNSLRAEDTAVYYCARGGYDTRNAMDYWGQGTTVTVSS

SEQ ID NO: 25 - protein, 120 aa, Artificial Sequence
  DOMAIN: VH2
EVQLVESGGGLVQPGGSLRLSCAASGFTFSDYGIHWVRQAPGKGLEWVAYISRGSSTIYYADTVKGRFTISRDNAKNSLYLQMTSLRAEDTAVYYCARGGYDTRNAMDYWGQGTTVTVSS

SEQ ID NO: 26 - protein, 120 aa, Artificial Sequence
  DOMAIN: VH3
EVQLVESGGGLVQPGGSLRLSCAASGFTFSDYGIHWVRQAPGKGLEWIAYISRGSSTIYYADTVKGRFTISRDNAKNSLYLQMTSLRAEDTAVYYCARGGYDTRNAMDYWGQGTTVTVSS

SEQ ID NO: 27 - protein, 120 aa, Artificial Sequence
  DOMAIN: VH4
EVQLVESGGGLVQPGGSLRLSCAASGFTFSDYGIHWVRQAPGKGLEWVAYISRGSSTIYYADTVKGRFTMSRDNAKNSLYLQMTSLRAEDTAVYYCARGGYDTRNAMDYWGQGTTVTVSS

SEQ ID NO: 28 - protein, 113 aa, Artificial Sequence
  DOMAIN: VL11
DIVMTQSPDSLAVSLGERATINCKSSQSLLNSGNQKNYLTWYQQKPGQPPKLLIYWASTRESGVPDRFSGSGSGTDFTLTISSLQAEDVAVYYCQNAYTYPFTFGQGTKLEIK

SEQ ID NO: 29 - protein, 113 aa, Artificial Sequence
  DOMAIN: VL12
DIVLTQSPDSLAVSLGERATINCKSSQSLLNSGNQKNYLTWYQQKPGQPPKLLIYWASTRESGVPDRFSGSGSGTDFTLTISSLQAEDVAVYYCQNAYTYPFTFGQGTKLEIK

SEQ ID NO: 30 - protein, 113 aa, Artificial Sequence
  DOMAIN: VL13
DIVLTQSPDSLAVSLGERATISCKSSQSLLNSGNQKNYLTWYQQKPGQPPKLLIYWASTRESGVPDRFSGSGSGTDFTLTISSLQAEDVAVYYCQNAYTYPFTFGQGTKLEIK

SEQ ID NO: 31 - protein, 118 aa, Artificial Sequence
  DOMAIN: VH11
EVQLVQSGAEVKKPGASVKVSCKASGYTFTSYWMHWVRQAPGQRLEWMGMIHPNSGSTNYNEKFKGRVTITRDTSASTAYMELSSLRSEDTAVYYCARLKTGNSFDYWGQGTTVTVSS

SEQ ID NO: 32 - protein, 118 aa, Artificial Sequence
  DOMAIN: VH12
EVQLVQSGAEVKKPGASVKVSCKASGYTFTSYWMHWVRQAPGQRLEWMGMIHPNSGSTNYNEKFKGRVTLTLDKSASTAYMELSSLRSEDTAVYYCARLKTGNSFDYWGQGTTVTVSS

SEQ ID NO: 33 - protein, 118 aa, Artificial Sequence
  DOMAIN: VH13
EVQLVQSGAEVKKPGASVKVSCKASGYTFTSYWMHWVRQAPGQRLEWIGMIHPNSGSTNYNEKFKGKATLTLDKSASTAYMELSSLRSEDTAVYYCARLKTGNSFDYWGQGTTVTVSS

SEQ ID NO: 34 - protein, 118 aa, Artificial Sequence
  DOMAIN: VH14
EVQLVQSGAEVKKPGASVKVSCKASGYTFTSYWMHWVKQRPGQRLEWIGMIHPNSGSTNYNEKFKGKATLTLDKSASTAYMELSSLRSEDTAVYYCARLKTGNSFDYWGQGTTVTVSS

SEQ ID NO: 35 - protein, 450 aa, Artificial Sequence
  CHAIN: ch1901 heavy chain
EVQLMESGGGLVKPGGSLKLSCAASGFTFSDYGIHWVRQAPEMGLEWIAYISRGSSTIYYADTVKGRFTMSRDNAKNTLFLQMTSLRSEDTAMYYCARGGYDTRNAMDYWGQGTSVTVSSASTKGPSVFPLAPSSKSTSGGTAALGCLVKDYFPEPVTVSWNSGALTSGVHTFPAVLQSSGLYSLSSVVTVPSSSLGTQTYICNVNHKPSNTKVDKKVEPKSCDKTHTCPPCPAPELLGGPSVFLFPPKPKDTLMISRTPEVTCVVVDVSHEDPEVKFNWYVDGVEVHNAKTKPREEQYNSTYRVVSVLTVLHQDWLNGKEYKCKVSNKALPAPIEKTISKAKGQPREPQVYTLPPSRDELTKNQVSLTCLVKGFYPSDIAVEWESNGQPENNYKTTPPVLDSDGSFFLYSKLTVDKSRWQQGNVFSCSVMHEALHNHYTQKSLSLSPGK

SEQ ID NO: 36 - protein, 220 aa, Artificial Sequence
  CHAIN: ch1901 light chain
DIVMTQSPSSLSVSAGEKVTMSCKSSQSLLNSGNQKNYLAWYQQKPGQPPKLLIYGASTRASGVPDRFTGSGSGTDFTLTISSVQAEDLAIYHCQNDLYYPLTFGAGTKLELKRTVAAPSVFIFPPSDEQLKSGTASVVCLLNNFYPREAKVQWKVDNALQSGNSQESVTEQDSKDSTYSLSSTLTLSKADYEKHKVYACEVTHQGLSSPVTKSFNRGEC

SEQ ID NO: 37 - protein, 448 aa, Artificial Sequence
  CHAIN: ch1902 heavy chain
EVQLQESGAELVKPGASVKLSCKASGYIFTSYWMHWVKQRPGQGLEWIGMIHPNSGSTNYNEKFKGKATLTLDKSSSTAYMQLSSLPSEDSAVYYCARLKTGNSFDYWGQGTTLTVSSASTKGPSVFPLAPSSKSTSGGTAALGCLVKDYFPEPVTVSWNSGALTSGVHTFPAVLQSSGLYSLSSVVTVPSSSLGTQTYICNVNHKPSNTKVDKKVEPKSCDKTHTCPPCPAPELLGGPSVFLFPPKPKDTLMISRTPEVTCVVVDVSHEDPEVKFNWYVDGVEVHNAKTKPREEQYNSTYRVVSVLTVLHQDWLNGKEYKCKVSNKALPAPIEKTISKAKGQPREPQVYTLPPSRDELTKNQVSLTCLVKGFYPSDIAVEWESNGQPENNYKTTPPVLDSDGSFFLYSKLTVDKSRWQQGNVFSCSVMHEALHNHYTQKSLSLSPGK

SEQ ID NO: 38 - protein, 220 aa, Artificial Sequence
  CHAIN: ch1902 light chain
DIVLTQSPSSLTVTAGEKVTMSCKSSQSLLNSGNQKNYLTWYQQKPGQPPKLLIYWASTRESGVPDRFTGSGSGTDFTLTISSVQAEDLAIYYCQNAYTYPFTFGSGTKLEIKRTVAAPSVFIFPPSDEQLKSGTASVVCLLNNFYPREAKVQWKVDNALQSGNSQESVTEQDSKDSTYSLSSTLTLSKADYEKHKVYACEVTHQGLSSPVTKSFNRGEC

SEQ ID NO: 39 - protein, 220 aa, Artificial Sequence
  CHAIN: L1
DIVMTQSPDSLAVSLGERATINCKSSQSLLNSGNQKNYLAWYQQKPGQPPKLLIYGASTRASGVPDRFSGSGSGTDFTLTISSLQAEDVAVYYCQNDLYYPLTFGQGTKLEIKRTVAAPSVFIFPPSDEQLKSGTASVVCLLNNFYPREAKVQWKVDNALQSGNSQESVTEQDSKDSTYSLSSTLTLSKADYEKHKVYACEVTHQGLSSPVTKSFNRGEC

SEQ ID NO: 40 - protein, 220 aa, Artificial Sequence
  CHAIN: L2
DIVMTQSPDSLAVSLGERATISCKSSQSLLNSGNQKNYLAWYQQKPGQPPKLLIYGASTRASGVPDRFSGSGSGTDFTLTISSLQAEDVAVYYCQNDLYYPLTFGQGTKLEIKRTVAAPSVFIFPPSDEQLKSGTASVVCLLNNFYPREAKVQWKVDNALQSGNSQESVTEQDSKDSTYSLSSTLTLSKADYEKHKVYACEVTHQGLSSPVTKSFNRGEC

SEQ ID NO: 41 - protein, 220 aa, Artificial Sequence
  CHAIN: L3
DIVMTQSPDSLAVSLGERATISCKSSQSLLNSGNQKNYLAWYQQKPGQPPKLLIYGASTRASGVPDRFSGSGSGTDFTLTISSLQAEDVAIYHCQNDLYYPLTFGQGTKLEIKRTVAAPSVFIFPPSDEQLKSGTASVVCLLNNFYPREAKVQWKVDNALQSGNSQESVTEQDSKDSTYSLSSTLTLSKADYEKHKVYACEVTHQGLSSPVTKSFNRGEC

SEQ ID NO: 42 - protein, 450 aa, Artificial Sequence
  CHAIN: H1
EVQLVESGGGLVQPGGSLRLSCAASGFTFSDYGIHWVRQAPGKGLEWVAYISRGSSTIYYADTVKGRFTISRDNAKNSLYLQMNSLRAEDTAVYYCARGGYDTRNAMDYWGQGTTVTVSSASTKGPSVFPLAPSSKSTSGGTAALGCLVKDYFPEPVTVSWNSGALTSGVHTFPAVLQSSGLYSLSSVVTVPSSSLGTQTYICNVNHKPSNTKVDKKVEPKSCDKTHTCPPCPAPELLGGPSVFLFPPKPKDTLMISRTPEVTCVVVDVSHEDPEVKFNWYVDGVEVHNAKTKPREEQYNSTYRVVSVLTVLHQDWLNGKEYKCKVSNKALPAPIEKTISKAKGQPREPQVYTLPPSRDELTKNQVSLTCLVKGFYPSDIAVEWESNGQPENNYKTTPPVLDSDGSFFLYSKLTVDKSRWQQGNVFSCSVMHEALHNHYTQKSLSLSPGK

SEQ ID NO: 43 - protein, 450 aa, Artificial Sequence
  CHAIN: H2
EVQLVESGGGLVQPGGSLRLSCAASGFTFSDYGIHWVRQAPGKGLEWVAYISRGSSTIYYADTVKGRFTISRDNAKNSLYLQMTSLRAEDTAVYYCARGGYDTRNAMDYWGQGTTVTVSSASTKGPSVFPLAPSSKSTSGGTAALGCLVKDYFPEPVTVSWNSGALTSGVHTFPAVLQSSGLYSLSSVVTVPSSSLGTQTYICNVNHKPSNTKVDKKVEPKSCDKTHTCPPCPAPELLGGPSVFLFPPKPKDTLMISRTPEVTCVVVDVSHEDPEVKFNWYVDGVEVHNAKTKPREEQYNSTYRVVSVLTVLHQDWLNGKEYKCKVSNKALPAPIEKTISKAKGQPREPQVYTLPPSRDELTKNQVSLTCLVKGFYPSDIAVEWESNGQPENNYKTTPPVLDSDGSFFLYSKLTVDKSRWQQGNVFSCSVMHEALHNHYTQKSLSLSPGK

SEQ ID NO: 44 - protein, 450 aa, Artificial Sequence
  CHAIN: H3
EVQLVESGGGLVQPGGSLRLSCAASGFTFSDYGIHWVRQAPGKGLEWIAYISRGSSTIYYADTVKGRFTISRDNAKNSLYLQMTSLRAEDTAVYYCARGGYDTRNAMDYWGQGTTVTVSSASTKGPSVFPLAPSSKSTSGGTAALGCLVKDYFPEPVTVSWNSGALTSGVHTFPAVLQSSGLYSLSSVVTVPSSSLGTQTYICNVNHKPSNTKVDKKVEPKSCDKTHTCPPCPAPELLGGPSVFLFPPKPKDTLMISRTPEVTCVVVDVSHEDPEVKFNWYVDGVEVHNAKTKPREEQYNSTYRVVSVLTVLHQDWLNGKEYKCKVSNKALPAPIEKTISKAKGQPREPQVYTLPPSRDELTKNQVSLTCLVKGFYPSDIAVEWESNGQPENNYKTTPPVLDSDGSFFLYSKLTVDKSRWQQGNVFSCSVMHEALHNHYTQKSLSLSPGK

SEQ ID NO: 45 - protein, 450 aa, Artificial Sequence
  CHAIN: H4
EVQLVESGGGLVQPGGSLRLSCAASGFTFSDYGIHWVRQAPGKGLEWVAYISRGSSTIYYADTVKGRFTMSRDNAKNSLYLQMTSLRAEDTAVYYCARGGYDTRNAMDYWGQGTTVTVSSASTKGPSVFPLAPSSKSTSGGTAALGCLVKDYFPEPVTVSWNSGALTSGVHTFPAVLQSSGLYSLSSVVTVPSSSLGTQTYICNVNHKPSNTKVDKKVEPKSCDKTHTCPPCPAPELLGGPSVFLFPPKPKDTLMISRTPEVTCVVVDVSHEDPEVKFNWYVDGVEVHNAKTKPREEQYNSTYRVVSVLTVLHQDWLNGKEYKCKVSNKALPAPIEKTISKAKGQPREPQVYTLPPSRDELTKNQVSLTCLVKGFYPSDIAVEWESNGQPENNYKTTPPVLDSDGSFFLYSKLTVDKSRWQQGNVFSCSVMHEALHNHYTQKSLSLSPGK

SEQ ID NO: 46 - protein, 220 aa, Artificial Sequence
  CHAIN: L11
DIVMTQSPDSLAVSLGERATINCKSSQSLLNSGNQKNYLTWYQQKPGQPPKLLIYWASTRESGVPDRFSGSGSGTDFTLTISSLQAEDVAVYYCQNAYTYPFTFGQGTKLEIKRTVAAPSVFIFPPSDEQLKSGTASVVCLLNNFYPREAKVQWKVDNALQSGNSQESVTEQDSKDSTYSLSSTLTLSKADYEKHKVYACEVTHQGLSSPVTKSFNRGEC

SEQ ID NO: 47 - protein, 220 aa, Artificial Sequence
  CHAIN: L12
DIVLTQSPDSLAVSLGERATINCKSSQSLLNSGNQKNYLTWYQQKPGQPPKLLIYWASTRESGVPDRFSGSGSGTDFTLTISSLQAEDVAVYYCQNAYTYPFTFGQGTKLEIKRTVAAPSVFIFPPSDEQLKSGTASVVCLLNNFYPREAKVQWKVDNALQSGNSQESVTEQDSKDSTYSLSSTLTLSKADYEKHKVYACEVTHQGLSSPVTKSFNRGEC

SEQ ID NO: 48 - protein, 220 aa, Artificial Sequence
  CHAIN: L13
DIVLTQSPDSLAVSLGERATISCKSSQSLLNSGNQKNYLTWYQQKPGQPPKLLIYWASTRESGVPDRFSGSGSGTDFTLTISSLQAEDVAVYYCQNAYTYPFTFGQGTKLEIKRTVAAPSVFIFPPSDEQLKSGTASVVCLLNNFYPREAKVQWKVDNALQSGNSQESVTEQDSKDSTYSLSSTLTLSKADYEKHKVYACEVTHQGLSSPVTKSFNRGEC

SEQ ID NO: 49 - protein, 448 aa, Artificial Sequence
  CHAIN: H11
EVQLVQSGAEVKKPGASVKVSCKASGYTFTSYWMHWVRQAPGQRLEWMGMIHPNSGSTNYNEKFKGRVTITRDTSASTAYMELSSLRSEDTAVYYCARLKTGNSFDYWGQGTTVTVSSASTKGPSVFPLAPSSKSTSGGTAALGCLVKDYFPEPVTVSWNSGALTSGVHTFPAVLQSSGLYSLSSVVTVPSSSLGTQTYICNVNHKPSNTKVDKKVEPKSCDKTHTCPPCPAPELLGGPSVFLFPPKPKDTLMISRTPEVTCVVVDVSHEDPEVKFNWYVDGVEVHNAKTKPREEQYNSTYRVVSVLTVLHQDWLNGKEYKCKVSNKALPAPIEKTISKAKGQPREPQVYTLPPSRDELTKNQVSLTCLVKGFYPSDIAVEWESNGQPENNYKTTPPVLDSDGSFFLYSKLTVDKSRWQQGNVFSCSVMHEALHNHYTQKSLSLSPGK

SEQ ID NO: 50 - protein, 448 aa, Artificial Sequence
  CHAIN: H12
EVQLVQSGAEVKKPGASVKVSCKASGYTFTSYWMHWVRQAPGQRLEWMGMIHPNSGSTNYNEKFKGRVTLTLDKSASTAYMELSSLRSEDTAVYYCARLKTGNSFDYWGQGTTVTVSSASTKGPSVFPLAPSSKSTSGGTAALGCLVKDYFPEPVTVSWNSGALTSGVHTFPAVLQSSGLYSLSSVVTVPSSSLGTQTYICNVNHKPSNTKVDKKVEPKSCDKTHTCPPCPAPELLGGPSVFLFPPKPKDTLMISRTPEVTCVVVDVSHEDPEVKFNWYVDGVEVHNAKTKPREEQYNSTYRVVSVLTVLHQDWLNGKEYKCKVSNKALPAPIEKTISKAKGQPREPQVYTLPPSRDELTKNQVSLTCLVKGFYPSDIAVEWESNGQPENNYKTTPPVLDSDGSFFLYSKLTVDKSRWQQGNVFSCSVMHEALHNHYTQKSLSLSPGK

SEQ ID NO: 51 - protein, 448 aa, Artificial Sequence
  CHAIN: H13
EVQLVQSGAEVKKPGASVKVSCKASGYTFTSYWMHWVRQAPGQRLEWIGMIHPNSGSTNYNEKFKGKATLTLDKSASTAYMELSSLRSEDTAVYYCARLKTGNSFDYWGQGTTVTVSSASTKGPSVFPLAPSSKSTSGGTAALGCLVKDYFPEPVTVSWNSGALTSGVHTFPAVLQSSGLYSLSSVVTVPSSSLGTQTYICNVNHKPSNTKVDKKVEPKSCDKTHTCPPCPAPELLGGPSVFLFPPKPKDTLMISRTPEVTCVVVDVSHEDPEVKFNWYVDGVEVHNAKTKPREEQYNSTYRVVSVLTVLHQDWLNGKEYKCKVSNKALPAPIEKTISKAKGQPREPQVYTLPPSRDELTKNQVSLTCLVKGFYPSDIAVEWESNGQPENNYKTTPPVLDSDGSFFLYSKLTVDKSRWQQGNVFSCSVMHEALHNHYTQKSLSLSPGK

SEQ ID NO: 52 - protein, 448 aa, Artificial Sequence
  CHAIN: H14
EVQLVQSGAEVKKPGASVKVSCKASGYTFTSYWMHWVKQRPGQRLEWIGMIHPNSGSTNYNEKFKGKATLTLDKSASTAYMELSSLRSEDTAVYYCARLKTGNSFDYWGQGTTVTVSSASTKGPSVFPLAPSSKSTSGGTAALGCLVKDYFPEPVTVSWNSGALTSGVHTFPAVLQSSGLYSLSSVVTVPSSSLGTQTYICNVNHKPSNTKVDKKVEPKSCDKTHTCPPCPAPELLGGPSVFLFPPKPKDTLMISRTPEVTCVVVDVSHEDPEVKFNWYVDGVEVHNAKTKPREEQYNSTYRVVSVLTVLHQDWLNGKEYKCKVSNKALPAPIEKTISKAKGQPREPQVYTLPPSRDELTKNQVSLTCLVKGFYPSDIAVEWESNGQPENNYKTTPPVLDSDGSFFLYSKLTVDKSRWQQGNVFSCSVMHEALHNHYTQKSLSLSPGK

SEQ ID NO: 53 - protein, 448 aa, Artificial Sequence
  CHAIN: IMAB-362 heavy chain
QVQLQQPGAELVRPGASVKLSCKASGYTFTSYWINWVKQRPGQGLEWIGNIYPSDSYTNYNQKFKDKATLTVDKSSSTAYMQLSSPTSEDSAVYYCTRSWRGNSFDYWGQGTTLTVSSASTKGPSVFPLAPSSKSTSGGTAALGCLVKDYFPEPVTVSWNSGALTSGVHTFPAVLQSSGLYSLSSVVTVPSSSLGTQTYICNVNHKPSNTKVDKRVEPKSCDKTHTCPPCPAPELLGGPSVFLFPPKPKDTLMISRTPEVTCVVVDVSHEDPEVKFNWYVDGVEVHNAKTKPREEQYNSTYRVVSVLTVLHQDWLNGKEYKCKVSNKALPAPIEKTISKAKGQPREPQVYTLPPSREEMTKNQVSLTCLVKGFYPSDIAVEWESNGQPENNYKTTPPVLDSDGSFFLYSKLTVDKSRWQQGNVFSCSVMHEALHNHYTQKSLSLSPGK

SEQ ID NO: 54 - protein, 220 aa, Artificial Sequence
  CHAIN: IMAB-362 light chain
DIVMTQSPSSLTVTAGEKVTMSCKSSQSLLNSGNQKNYLTWYQQKPGQPPKLLIYWASTRESGVPDRFTGSGSGTDFTLTISSVQAEDLAVYYCQNDYSYPFTFGSGTKLEIKRTVAAPSVFIFPPSDEQLKSGTASVVCLLNNFYPREAKVQWKVDNALQSGNSQESVTEQDSKDSTYSLSSTLTLSKADYEKHKVYACEVTHQGLSSPVTKSFNRGEC

SEQ ID NO: 55 - protein, 18 aa, Artificial Sequence
  PEPTIDE: Signal peptide
  UNSURE (16)..(16): Xaa is Val, Ala, Ser, Thr, Gly, Cys, Leu or Ile
  UNSURE (18)..(18): Xaa is Ala, Gly, Ser, Cys, Thr or Gln
MEWSWVFLFFLSLTGXHX

SEQ ID NO: 56 - protein, 20 aa, Artificial Sequence
  PEPTIDE: Signal peptide
  UNSURE (18)..(18): Xaa is Val, Ala, Ser, Thr, Gly, Cys, Leu or Ile
  UNSURE (20)..(20): Xaa is Ala, Gly, Ser, Cys, Thr or Gln
  UNSURE (20)..(20): When Xaa(18) is Ala, Xaa(20) is not Cys
MSVPTQVLGLLLLWLTDXRX

SEQ ID NO: 57 - protein, 18 aa, Artificial Sequence
  PEPTIDE: Signal peptide
MEWSWVFLFFLSLTGVHA

SEQ ID NO: 58 - protein, 18 aa, Artificial Sequence
  PEPTIDE: Signal peptide
MEWSWVFLFFLSLTGVHG

SEQ ID NO: 59 - protein, 18 aa, Artificial Sequence
  PEPTIDE: Signal peptide
MEWSWVFLFFLSLTGVHS

SEQ ID NO: 60 - protein, 18 aa, Artificial Sequence
  PEPTIDE: Signal peptide
MEWSWVFLFFLSLTGVHC

SEQ ID NO: 61 - protein, 18 aa, Artificial Sequence
  PEPTIDE: Signal peptide
MEWSWVFLFFLSLTGVHT

SEQ ID NO: 62 - protein, 18 aa, Artificial Sequence
  PEPTIDE: Signal peptide
MEWSWVFLFFLSLTGVHQ

SEQ ID NO: 63 - protein, 18 aa, Artificial Sequence
  PEPTIDE: Signal peptide
MEWSWVFLFFLSLTGAHA

SEQ ID NO: 64 - protein, 18 aa, Artificial Sequence
  PEPTIDE: Signal peptide
MEWSWVFLFFLSLTGAHG

SEQ ID NO: 65 - protein, 18 aa, Artificial Sequence
  PEPTIDE: Signal peptide
MEWSWVFLFFLSLTGAHS

SEQ ID NO: 66 - protein, 18 aa, Artificial Sequence
  PEPTIDE: Signal peptide
MEWSWVFLFFLSLTGAHC

SEQ ID NO: 67 - protein, 18 aa, Artificial Sequence
  PEPTIDE: Signal peptide
MEWSWVFLFFLSLTGAHT

SEQ ID NO: 68 - protein, 18 aa, Artificial Sequence
  PEPTIDE: Signal peptide
MEWSWVFLFFLSLTGAHQ

SEQ ID NO: 69 - protein, 18 aa, Artificial Sequence
  PEPTIDE: Signal peptide
MEWSWVFLFFLSLTGSHA

SEQ ID NO: 70 - protein, 18 aa, Artificial Sequence
  PEPTIDE: Signal peptide
MEWSWVFLFFLSLTGSHG

SEQ ID NO: 71 - protein, 18 aa, Artificial Sequence
  PEPTIDE: Signal peptide
MEWSWVFLFFLSLTGSHS

SEQ ID NO: 72 - protein, 18 aa, Artificial Sequence
  PEPTIDE: Signal peptide
MEWSWVFLFFLSLTGSHC

SEQ ID NO: 73 - protein, 18 aa, Artificial Sequence
  PEPTIDE: Signal peptide
MEWSWVFLFFLSLTGSHT

SEQ ID NO: 74 - protein, 18 aa, Artificial Sequence
  PEPTIDE: Signal peptide
MEWSWVFLFFLSLTGSHQ

SEQ ID NO: 75 - protein, 18 aa, Artificial Sequence
  PEPTIDE: Signal peptide
MEWSWVFLFFLSLTGTHA

SEQ ID NO: 76 - protein, 18 aa, Artificial Sequence
  PEPTIDE: Signal peptide
MEWSWVFLFFLSLTGTHG

SEQ ID NO: 77 - protein, 18 aa, Artificial Sequence
  PEPTIDE: Signal peptide
MEWSWVFLFFLSLTGTHS

SEQ ID NO: 78 - protein, 18 aa, Artificial Sequence
  PEPTIDE: Signal peptide
MEWSWVFLFFLSLTGTHC

SEQ ID NO: 79 - protein, 18 aa, Artificial Sequence
  PEPTIDE: Signal peptide
MEWSWVFLFFLSLTGTHT

SEQ ID NO: 80 - protein, 18 aa, Artificial Sequence
  PEPTIDE: Signal peptide
MEWSWVFLFFLSLTGTHQ

SEQ ID NO: 81 - protein, 18 aa, Artificial Sequence
  PEPTIDE: Signal peptide
MEWSWVFLFFLSLTGGHA

SEQ ID NO: 82 - protein, 18 aa, Artificial Sequence
  PEPTIDE: Signal peptide
MEWSWVFLFFLSLTGGHG

SEQ ID NO: 83 - protein, 18 aa, Artificial Sequence
  PEPTIDE: Signal peptide
MEWSWVFLFFLSLTGGHS

SEQ ID NO: 84 - protein, 18 aa, Artificial Sequence
  PEPTIDE: Signal peptide
MEWSWVFLFFLSLTGGHC

SEQ ID NO: 85 - protein, 18 aa, Artificial Sequence
  PEPTIDE: Signal peptide
MEWSWVFLFFLSLTGGHT

SEQ ID NO: 86 - protein, 18 aa, Artificial Sequence
  PEPTIDE: Signal peptide
MEWSWVFLFFLSLTGGHQ

SEQ ID NO: 87 - protein, 18 aa, Artificial Sequence
  PEPTIDE: Signal peptide
MEWSWVFLFFLSLTGCHA

SEQ ID NO: 88 - protein, 18 aa, Artificial Sequence
  PEPTIDE: Signal peptide
MEWSWVFLFFLSLTGCHG

SEQ ID NO: 89 - protein, 18 aa, Artificial Sequence
  PEPTIDE: Signal peptide
MEWSWVFLFFLSLTGCHS

SEQ ID NO: 90 - protein, 18 aa, Artificial Sequence
  PEPTIDE: Signal peptide
MEWSWVFLFFLSLTGCHC

SEQ ID NO: 91 - protein, 18 aa, Artificial Sequence
  PEPTIDE: Signal peptide
MEWSWVFLFFLSLTGCHT

SEQ ID NO: 92 - protein, 18 aa, Artificial Sequence
  PEPTIDE: Signal peptide
MEWSWVFLFFLSLTGCHQ

SEQ ID NO: 93 - protein, 18 aa, Artificial Sequence
  PEPTIDE: Signal peptide
MEWSWVFLFFLSLTGLHA

SEQ ID NO: 94 - protein, 18 aa, Artificial Sequence
  PEPTIDE: Signal peptide
MEWSWVFLFFLSLTGLHG

SEQ ID NO: 95 - protein, 18 aa, Artificial Sequence
  PEPTIDE: Signal peptide
MEWSWVFLFFLSLTGLHS

SEQ ID NO: 96 - protein, 18 aa, Artificial Sequence
  PEPTIDE: Signal peptide
MEWSWVFLFFLSLTGLHC

SEQ ID NO: 97 - protein, 18 aa, Artificial Sequence
  PEPTIDE: Signal peptide
MEWSWVFLFFLSLTGLHT

SEQ ID NO: 98 - protein, 18 aa, Artificial Sequence
  PEPTIDE: Signal peptide
MEWSWVFLFFLSLTGLHQ

SEQ ID NO: 99 - protein, 18 aa, Artificial Sequence
  PEPTIDE: Signal peptide
MEWSWVFLFFLSLTGIHA

SEQ ID NO: 100 - protein, 18 aa, Artificial Sequence
  PEPTIDE: Signal peptide
MEWSWVFLFFLSLTGIHG

SEQ ID NO: 101 - protein, 18 aa, Artificial Sequence
  PEPTIDE: Signal peptide
MEWSWVFLFFLSLTGIHS

SEQ ID NO: 102 - protein, 18 aa, Artificial Sequence
  PEPTIDE: Signal peptide
MEWSWVFLFFLSLTGIHC

SEQ ID NO: 103 - protein, 18 aa, Artificial Sequence
  PEPTIDE: Signal peptide
MEWSWVFLFFLSLTGIHT

SEQ ID NO: 104 - protein, 18 aa, Artificial Sequence
  PEPTIDE: Signal peptide
MEWSWVFLFFLSLTGIHQ

SEQ ID NO: 105 - protein, 20 aa, Artificial Sequence
  PEPTIDE: Signal peptide
MSVPTQVLGLLLLWLTDVRA

SEQ ID NO: 106 - protein, 20 aa, Artificial Sequence
  PEPTIDE: Signal peptide
MSVPTQVLGLLLLWLTDVRG

SEQ ID NO: 107 - protein, 20 aa, Artificial Sequence
  PEPTIDE: Signal peptide
MSVPTQVLGLLLLWLTDVRS

SEQ ID NO: 108 - protein, 20 aa, Artificial Sequence
  PEPTIDE: Signal peptide
MSVPTQVLGLLLLWLTDVRC

SEQ ID NO: 109 - protein, 20 aa, Artificial Sequence
  PEPTIDE: Signal peptide
MSVPTQVLGLLLLWLTDVRT

SEQ ID NO: 110 - protein, 20 aa, Artificial Sequence
  PEPTIDE: Signal peptide
MSVPTQVLGLLLLWLTDVRQ

SEQ ID NO: 111 - protein, 20 aa, Artificial Sequence
  PEPTIDE: Signal peptide
MSVPTQVLGLLLLWLTDARA

SEQ ID NO: 112 - protein, 20 aa, Artificial Sequence
  PEPTIDE: Signal peptide
MSVPTQVLGLLLLWLTDARG

SEQ ID NO: 113 - protein, 20 aa, Artificial Sequence
  PEPTIDE: Signal peptide
MSVPTQVLGLLLLWLTDARS

SEQ ID NO: 114 - protein, 20 aa, Artificial Sequence
  PEPTIDE: Signal peptide
MSVPTQVLGLLLLWLTDART

SEQ ID NO: 115 - protein, 20 aa, Artificial Sequence
  PEPTIDE: Signal peptide
MSVPTQVLGLLLLWLTDARQ

SEQ ID NO: 116 - protein, 20 aa, Artificial Sequence
  PEPTIDE: Signal peptide
MSVPTQVLGLLLLWLTDSRA

SEQ ID NO: 117 - protein, 20 aa, Artificial Sequence
  PEPTIDE: Signal peptide
MSVPTQVLGLLLLWLTDSRG

SEQ ID NO: 118 - protein, 20 aa, Artificial Sequence
  PEPTIDE: Signal peptide
MSVPTQVLGLLLLWLTDSRS

SEQ ID NO: 119 - protein, 20 aa, Artificial Sequence
  PEPTIDE: Signal peptide
MSVPTQVLGLLLLWLTDSRC

SEQ ID NO: 120 - protein, 20 aa, Artificial Sequence
  PEPTIDE: Signal peptide
MSVPTQVLGLLLLWLTDSRT

SEQ ID NO: 121 - protein, 20 aa, Artificial Sequence
  PEPTIDE: Signal peptide
MSVPTQVLGLLLLWLTDSRQ

SEQ ID NO: 122 - protein, 20 aa, Artificial Sequence
  PEPTIDE: Signal peptide
MSVPTQVLGLLLLWLTDTRA

SEQ ID NO: 123 - protein, 20 aa, Artificial Sequence
  PEPTIDE: Signal peptide
MSVPTQVLGLLLLWLTDTRG

SEQ ID NO: 124 - protein, 20 aa, Artificial Sequence
  PEPTIDE: Signal peptide
MSVPTQVLGLLLLWLTDTRS

SEQ ID NO: 125 - protein, 20 aa, Artificial Sequence
  PEPTIDE: Signal peptide
MSVPTQVLGLLLLWLTDTRC

SEQ ID NO: 126 - protein, 20 aa, Artificial Sequence
  PEPTIDE: Signal peptide
MSVPTQVLGLLLLWLTDTRT

SEQ ID NO: 127 - protein, 20 aa, Artificial Sequence
  PEPTIDE: Signal peptide
MSVPTQVLGLLLLWLTDTRQ

SEQ ID NO: 128 - protein, 20 aa, Artificial Sequence
  PEPTIDE: Signal peptide
MSVPTQVLGLLLLWLTDGRA

SEQ ID NO: 129 - protein, 20 aa, Artificial Sequence
  PEPTIDE: Signal peptide
MSVPTQVLGLLLLWLTDGRG

SEQ ID NO: 130 - protein, 20 aa, Artificial Sequence
  PEPTIDE: Signal peptide
MSVPTQVLGLLLLWLTDGRS

SEQ ID NO: 131 - protein, 20 aa, Artificial Sequence
  PEPTIDE: Signal peptide
MSVPTQVLGLLLLWLTDGRC

SEQ ID NO: 132 - protein, 20 aa, Artificial Sequence
  PEPTIDE: Signal peptide
MSVPTQVLGLLLLWLTDGRT

SEQ ID NO: 133 - protein, 20 aa, Artificial Sequence
  PEPTIDE: Signal peptide
MSVPTQVLGLLLLWLTDGRQ

SEQ ID NO: 134 - protein, 20 aa, Artificial Sequence
  PEPTIDE: Signal peptide
MSVPTQVLGLLLLWLTDCRA

SEQ ID NO: 135 - protein, 20 aa, Artificial Sequence
  PEPTIDE: Signal peptide
MSVPTQVLGLLLLWLTDCRG

SEQ ID NO: 136 - protein, 20 aa, Artificial Sequence
  PEPTIDE: Signal peptide
MSVPTQVLGLLLLWLTDCRS

SEQ ID NO: 137 - protein, 20 aa, Artificial Sequence
  PEPTIDE: Signal peptide
MSVPTQVLGLLLLWLTDCRC

SEQ ID NO: 138 - protein, 20 aa, Artificial Sequence
  PEPTIDE: Signal peptide
MSVPTQVLGLLLLWLTDCRT

SEQ ID NO: 139 - protein, 20 aa, Artificial Sequence
  PEPTIDE: Signal peptide
MSVPTQVLGLLLLWLTDCRQ

SEQ ID NO: 140 - protein, 20 aa, Artificial Sequence
  PEPTIDE: Signal peptide
MSVPTQVLGLLLLWLTDLRA

SEQ ID NO: 141 - protein, 20 aa, Artificial Sequence
  PEPTIDE: Signal peptide
MSVPTQVLGLLLLWLTDLRG

SEQ ID NO: 142 - protein, 20 aa, Artificial Sequence
  PEPTIDE: Signal peptide
MSVPTQVLGLLLLWLTDLRS

SEQ ID NO: 143 - protein, 20 aa, Artificial Sequence
  PEPTIDE: Signal peptide
MSVPTQVLGLLLLWLTDLRC

SEQ ID NO: 144 - protein, 20 aa, Artificial Sequence
  PEPTIDE: Signal peptide
MSVPTQVLGLLLLWLTDLRT

SEQ ID NO: 145 - protein, 20 aa, Artificial Sequence
  PEPTIDE: Signal peptide
MSVPTQVLGLLLLWLTDLRQ

SEQ ID NO: 146 - protein, 20 aa, Artificial Sequence
  PEPTIDE: Signal peptide
MSVPTQVLGLLLLWLTDIRA

SEQ ID NO: 147 - protein, 20 aa, Artificial Sequence
  PEPTIDE: Signal peptide
MSVPTQVLGLLLLWLTDIRG

SEQ ID NO: 148 - protein, 20 aa, Artificial Sequence
  PEPTIDE: Signal peptide
MSVPTQVLGLLLLWLTDIRS

SEQ ID NO: 149 - protein, 20 aa, Artificial Sequence
  PEPTIDE: Signal peptide
MSVPTQVLGLLLLWLTDIRC

SEQ ID NO: 150 - protein, 20 aa, Artificial Sequence
  PEPTIDE: Signal peptide
MSVPTQVLGLLLLWLTDIRT

SEQ ID NO: 151 - protein, 20 aa, Artificial Sequence
  PEPTIDE: Signal peptide
MSVPTQVLGLLLLWLTDIRQ

SEQ ID NO: 152 - protein, 19 aa, Artificial Sequence
  PEPTIDE: Signal peptide
MEWSWVFLFFLSVTTGVHS

SEQ ID NO: 153 - protein, 20 aa, Artificial Sequence
  PEPTIDE: Signal peptide
MSVPTQVLGLLLLWLTDARC

SEQ ID NO: 154 - protein, 468 aa, Artificial Sequence
  CHAIN: Pertuzumab-1 antibody heavy chain containing signal peptide
MEWSWVFLFFLSVTTGVHSEVQLVESGGGLVQPGGSLRLSCAASGFTFTDYTMDWVRQAPGKGLEWVADVNPNSGGSIYNQRFKGRFTLSVDRSKNTLYLQMNSLRAEDTAVYYCARNLGPSFYFDYWGQGTLVTVSSASTKGPSVFPLAPSSKSTSGGTAALGCLVKDYFPEPVTVSWNSGALTSGVHTFPAVLQSSGLYSLSSVVTVPSSSLGTQTYICNVNHKPSNTKVDKKVEPKSCDKTHTCPPCPAPELLGGPSVFLFPPKPKDTLMISRTPEVTCVVVDVSHEDPEVKFNWYVDGVEVHNAKTKPREEQYNSTYRVVSVLTVLHQDWLNGKEYKCKVSNKALPAPIEKTISKAKGQPREPQVYTLPPSREEMTKNQVSLTCLVKGFYPSDIAVEWESNGQPENNYKTTPPVLDSDGSFFLYSKLTVDKSRWQQGNVFSCSVMHEALHNHYTQKSLSLSPGK

SEQ ID NO: 155 - protein, 234 aa, Artificial Sequence
  CHAIN: Pertuzumab-1 antibody light chain containing signal peptide
MSVPTQVLGLLLLWLTDARCDIQMTQSPSSLSASVGDRVTITCKASQDVSIGVAWYQQKPGKAPKLLIYSASYRYTGVPSRFSGSGSGTDFTLTISSLQPEDFATYYCQQYYIYPYTFGQGTKVEIKRTVAAPSVFIFPPSDEQLKSGTASVVCLLNNFYPREAKVQWKVDNALQSGNSQESVTEQDSKDSTYSLSSTLTLSKADYEKHKVYACEVTHQGLSSPVTKSFNRGEC

SEQ ID NO: 156 - protein, 233 aa, Artificial Sequence
  CHAIN: Pertuzumab-2 antibody heavy chain containing signal peptide
MEWSWVFLFFLSVTTGVHSDIQMTQSPSSLSASVGDRVTITCKASQDVSIGVAWYQQKPGKAPKLLIYSASYRYTGVPSRFSGSGSGTDFTLTISSLQPEDFATYYCQQYYIYPYTFGQGTKVEIKRTVAAPSVFIFPPSDEQLKSGTASVVCLLNNFYPREAKVQWKVDNALQSGNSQESVTEQDSKDSTYSLSSTLTLSKADYEKHKVYACEVTHQGLSSPVTKSFNRGEC

SEQ ID NO: 157 - protein, 467 aa, Artificial Sequence
  CHAIN: Pertuzumab-3 antibody heavy chain containing signal peptide
MEWSWVFLFFLSLTGVHAEVQLVESGGGLVQPGGSLRLSCAASGFTFTDYTMDWVRQAPGKGLEWVADVNPNSGGSIYNQRFKGRFTLSVDRSKNTLYLQMNSLRAEDTAVYYCARNLGPSFYFDYWGQGTLVTVSSASTKGPSVFPLAPSSKSTSGGTAALGCLVKDYFPEPVTVSWNSGALTSGVHTFPAVLQSSGLYSLSSVVTVPSSSLGTQTYICNVNHKPSNTKVDKKVEPKSCDKTHTCPPCPAPELLGGPSVFLFPPKPKDTLMISRTPEVTCVVVDVSHEDPEVKFNWYVDGVEVHNAKTKPREEQYNSTYRVVSVLTVLHQDWLNGKEYKCKVSNKALPAPIEKTISKAKGQPREPQVYTLPPSREEMTKNQVSLTCLVKGFYPSDIAVEWESNGQPENNYKTTPPVLDSDGSFFLYSKLTVDKSRWQQGNVFSCSVMHEALHNHYTQKSLSLSPGK

SEQ ID NO: 158 - protein, 234 aa, Artificial Sequence
  CHAIN: Pertuzumab-3 antibody light chain containing signal peptide
MSVPTQVLGLLLLWLTDVRADIQMTQSPSSLSASVGDRVTITCKASQDVSIGVAWYQQKPGKAPKLLIYSASYRYTGVPSRFSGSGSGTDFTLTISSLQPEDFATYYCQQYYIYPYTFGQGTKVEIKRTVAAPSVFIFPPSDEQLKSGTASVVCLLNNFYPREAKVQWKVDNALQSGNSQESVTEQDSKDSTYSLSSTLTLSKADYEKHKVYACEVTHQGLSSPVTKSFNRGEC

SEQ ID NO: 159 - protein, 232 aa, Artificial Sequence
  CHAIN: Pertuzumab-4 antibody light chain containing signal peptide
MEWSWVFLFFLSLTGVHADIQMTQSPSSLSASVGDRVTITCKASQDVSIGVAWYQQKPGKAPKLLIYSASYRYTGVPSRFSGSGSGTDFTLTISSLQPEDFATYYCQQYYIYPYTFGQGTKVEIKRTVAAPSVFIFPPSDEQLKSGTASVVCLLNNFYPREAKVQWKVDNALQSGNSQESVTEQDSKDSTYSLSSTLTLSKADYEKHKVYACEVTHQGLSSPVTKSFNRGEC

SEQ ID NO: 160 - protein, 469 aa, Artificial Sequence
  CHAIN: Pertuzumab-5 antibody heavy chain containing signal peptide
MSVPTQVLGLLLLWLTDVRAEVQLVESGGGLVQPGGSLRLSCAASGFTFTDYTMDWVRQAPGKGLEWVADVNPNSGGSIYNQRFKGRFTLSVDRSKNTLYLQMNSLRAEDTAVYYCARNLGPSFYFDYWGQGTLVTVSSASTKGPSVFPLAPSSKSTSGGTAALGCLVKDYFPEPVTVSWNSGALTSGVHTFPAVLQSSGLYSLSSVVTVPSSSLGTQTYICNVNHKPSNTKVDKKVEPKSCDKTHTCPPCPAPELLGGPSVFLFPPKPKDTLMISRTPEVTCVVVDVSHEDPEVKFNWYVDGVEVHNAKTKPREEQYNSTYRVVSVLTVLHQDWLNGKEYKCKVSNKALPAPIEKTISKAKGQPREPQVYTLPPSREEMTKNQVSLTCLVKGFYPSDIAVEWESNGQPENNYKTTPPVLDSDGSFFLYSKLTVDKSRWQQGNVFSCSVMHEALHNHYTQKSLSLSPGK

SEQ ID NO: 161 - protein, 467 aa, Artificial Sequence
  CHAIN: h1902-5-1 antibody heavy chain containing signal peptide
MEWSWVFLFFLSVTTGVHSEVQLVQSGAEVKKPGASVKVSCKASGYTFTSYWMHWVRQAPGQRLEWMGMIHPNSGSTNYNEKFKGRVTITRDTSASTAYMELSSLRSEDTAVYYCARLKTGNSFDYWGQGTTVTVSSASTKGPSVFPLAPSSKSTSGGTAALGCLVKDYFPEPVTVSWNSGALTSGVHTFPAVLQSSGLYSLSSVVTVPSSSLGTQTYICNVNHKPSNTKVDKKVEPKSCDKTHTCPPCPAPELLGGPSVFLFPPKPKDTLMISRTPEVTCVVVDVSHEDPEVKFNWYVDGVEVHNAKTKPREEQYNSTYRVVSVLTVLHQDWLNGKEYKCKVSNKALPAPIEKTISKAKGQPREPQVYTLPPSRDELTKNQVSLTCLVKGFYPSDIAVEWESNGQPENNYKTTPPVLDSDGSFFLYSKLTVDKSRWQQGNVFSCSVMHEALHNHYTQKSLSLSPGK

SEQ ID NO: 162 - protein, 239 aa, Artificial Sequence
  CHAIN: h1902-5-1 antibody light chain containing signal peptide
MEWSWVFLFFLSVTTGVHSDIVLTQSPDSLAVSLGERATINCKSSQSLLNSGNQKNYLTWYQQKPGQPPKLLIYWASTRESGVPDRFSGSGSGTDFTLTISSLQAEDVAVYYCQNAYTYPFTFGQGTKLEIKRTVAAPSVFIFPPSDEQLKSGTASVVCLLNNFYPREAKVQWKVDNALQSGNSQESVTEQDSKDSTYSLSSTLTLSKADYEKHKVYACEVTHQGLSSPVTKSFNRGEC

SEQ ID NO: 163 - protein, 466 aa, Artificial Sequence
  CHAIN: h1902-5-2 antibody heavy chain containing signal peptide
MEWSWVFLFFLSLTGVHAEVQLVQSGAEVKKPGASVKVSCKASGYTFTSYWMHWVRQAPGQRLEWMGMIHPNSGSTNYNEKFKGRVTITRDTSASTAYMELSSLRSEDTAVYYCARLKTGNSFDYWGQGTTVTVSSASTKGPSVFPLAPSSKSTSGGTAALGCLVKDYFPEPVTVSWNSGALTSGVHTFPAVLQSSGLYSLSSVVTVPSSSLGTQTYICNVNHKPSNTKVDKKVEPKSCDKTHTCPPCPAPELLGGPSVFLFPPKPKDTLMISRTPEVTCVVVDVSHEDPEVKFNWYVDGVEVHNAKTKPREEQYNSTYRVVSVLTVLHQDWLNGKEYKCKVSNKALPAPIEKTISKAKGQPREPQVYTLPPSRDELTKNQVSLTCLVKGFYPSDIAVEWESNGQPENNYKTTPPVLDSDGSFFLYSKLTVDKSRWQQGNVFSCSVMHEALHNHYTQKSLSLSPGK

SEQ ID NO: 164 - protein, 240 aa, Artificial Sequence
  CHAIN: h1902-5-2 antibody light chain containing signal peptide
MSVPTQVLGLLLLWLTDVRADIVLTQSPDSLAVSLGERATINCKSSQSLLNSGNQKNYLTWYQQKPGQPPKLLIYWASTRESGVPDRFSGSGSGTDFTLTISSLQAEDVAVYYCQNAYTYPFTFGQGTKLEIKRTVAAPSVFIFPPSDEQLKSGTASVVCLLNNFYPREAKVQWKVDNALQSGNSQESVTEQDSKDSTYSLSSTLTLSKADYEKHKVYACEVTHQGLSSPVTKSFNRGEC

SEQ ID NO: 165 - protein, 468 aa, Artificial Sequence
  CHAIN: h1902-5-3 antibody heavy chain containing signal peptide
MSVPTQVLGLLLLWLTDVRAEVQLVQSGAEVKKPGASVKVSCKASGYTFTSYWMHWVRQAPGQRLEWMGMIHPNSGSTNYNEKFKGRVTITRDTSASTAYMELSSLRSEDTAVYYCARLKTGNSFDYWGQGTTVTVSSASTKGPSVFPLAPSSKSTSGGTAALGCLVKDYFPEPVTVSWNSGALTSGVHTFPAVLQSSGLYSLSSVVTVPSSSLGTQTYICNVNHKPSNTKVDKKVEPKSCDKTHTCPPCPAPELLGGPSVFLFPPKPKDTLMISRTPEVTCVVVDVSHEDPEVKFNWYVDGVEVHNAKTKPREEQYNSTYRVVSVLTVLHQDWLNGKEYKCKVSNKALPAPIEKTISKAKGQPREPQVYTLPPSRDELTKNQVSLTCLVKGFYPSDIAVEWESNGQPENNYKTTPPVLDSDGSFFLYSKLTVDKSRWQQGNVFSCSVMHEALHNHYTQKSLSLSPGK

SEQ ID NO: 166 - protein, 238 aa, Artificial Sequence
  CHAIN: h1902-5-3 antibody light chain containing signal peptide
MEWSWVFLFFLSLTGVHADIVLTQSPDSLAVSLGERATINCKSSQSLLNSGNQKNYLTWYQQKPGQPPKLLIYWASTRESGVPDRFSGSGSGTDFTLTISSLQAEDVAVYYCQNAYTYPFTFGQGTKLEIKRTVAAPSVFIFPPSDEQLKSGTASVVCLLNNFYPREAKVQWKVDNALQSGNSQESVTEQDSKDSTYSLSSTLTLSKADYEKHKVYACEVTHQGLSSPVTKSFNRGEC

SEQ ID NO: 167 - protein, 449 aa, Artificial Sequence
  CHAIN: Heavy chain of anti-FcRn antibody
EVQLVQSGAEVKKPGESLKISCKGSGYNFNKHYIAWVRQMPGKGLEWMGIIYPDNSNTIYSPSFQGQVTISADKSISTAYLQWSSLKASDTAMYYCARFGGPTFAQWYFDYWGQGTLVTVSSASTKGPSVFPLAPCSRSTSESTAALGCLVKDYFPEPVTVSWNSGALTSGVHTFPAVLQSSGLYSLSSVVTVPSSSLGTKTYTCNVDHKPSNTKVDKRVESKYGPPCPPCPAPEFLGGPSVFLFPPKPKDTLMISRTPEVTCVVVDVSQEDPEVQFNWYVDGVEVHNAKTKPREEQFNSTYRVVSVLTVLHQDWLNGKEYKCKVSNKGLPSSIEKTISKAKGQPREPQVYTLPPSQEEMTKNQVSLTCLVKGFYPSDIAVEWESNGQPENNYKTTPPVLDSDGSFFLYSRLTVDKSRWQEGNVFSCSVMHEALHNHYTQKSLSLSLGK

SEQ ID NO: 168 - protein, 218 aa, Artificial Sequence
  CHAIN: Light chain of anti-FcRn antibody
NFMLTQPHSVSESPGKTVTISCTGSSGSIASNYVQWYQQRPGSSPTTVIYEDNQRASGVPDRFSGSIDSSSNSASLTISGLKTEDEADYYCQSYDSSSHNWVFGGGTKLTVLGQPKANPTVTLFPPSSEELQANKATLVCLISDFYPGAVTVAWKADGSPVKAGVETTKPSKQSNNKYAASSYLSLTPEQWKSHRSYSCQVTHEGSTVEKTVAPTECS

SEQ ID NO: 169 - protein, 468 aa, Artificial Sequence
  CHAIN: Amino acid sequence of FcRn-1 antibody heavy chain containing signal peptide
MEWSWVFLFFLSVTTGVHSEVQLVQSGAEVKKPGESLKISCKGSGYNFNKHYIAWVRQMPGKGLEWMGIIYPDNSNTIYSPSFQGQVTISADKSISTAYLQWSSLKASDTAMYYCARFGGPTFAQWYFDYWGQGTLVTVSSASTKGPSVFPLAPCSRSTSESTAALGCLVKDYFPEPVTVSWNSGALTSGVHTFPAVLQSSGLYSLSSVVTVPSSSLGTKTYTCNVDHKPSNTKVDKRVESKYGPPCPPCPAPEFLGGPSVFLFPPKPKDTLMISRTPEVTCVVVDVSQEDPEVQFNWYVDGVEVHNAKTKPREEQFNSTYRVVSVLTVLHQDWLNGKEYKCKVSNKGLPSSIEKTISKAKGQPREPQVYTLPPSQEEMTKNQVSLTCLVKGFYPSDIAVEWESNGQPENNYKTTPPVLDSDGSFFLYSRLTVDKSRWQEGNVFSCSVMHEALHNHYTQKSLSLSLGK

SEQ ID NO: 170 - protein, 237 aa, Artificial Sequence
  CHAIN: Amino acid sequence of FcRn-1 antibody light chain containing signal peptide
MEWSWVFLFFLSVTTGVHSNFMLTQPHSVSESPGKTVTISCTGSSGSIASNYVQWYQQRPGSSPTTVIYEDNQRASGVPDRFSGSIDSSSNSASLTISGLKTEDEADYYCQSYDSSSHNWVFGGGTKLTVLGQPKANPTVTLFPPSSEELQANKATLVCLISDFYPGAVTVAWKADGSPVKAGVETTKPSKQSNNKYAASSYLSLTPEQWKSHRSYSCQVTHEGSTVEKTVAPTECS

SEQ ID NO: 171 - protein, 467 aa, Artificial Sequence
  CHAIN: Amino acid sequence of FcRn-2 antibody heavy chain containing signal peptide
MEWSWVFLFFLSLTGVHAEVQLVQSGAEVKKPGESLKISCKGSGYNFNKHYIAWVRQMPGKGLEWMGIIYPDNSNTIYSPSFQGQVTISADKSISTAYLQWSSLKASDTAMYYCARFGGPTFAQWYFDYWGQGTLVTVSSASTKGPSVFPLAPCSRSTSESTAALGCLVKDYFPEPVTVSWNSGALTSGVHTFPAVLQSSGLYSLSSVVTVPSSSLGTKTYTCNVDHKPSNTKVDKRVESKYGPPCPPCPAPEFLGGPSVFLFPPKPKDTLMISRTPEVTCVVVDVSQEDPEVQFNWYVDGVEVHNAKTKPREEQFNSTYRVVSVLTVLHQDWLNGKEYKCKVSNKGLPSSIEKTISKAKGQPREPQVYTLPPSQEEMTKNQVSLTCLVKGFYPSDIAVEWESNGQPENNYKTTPPVLDSDGSFFLYSRLTVDKSRWQEGNVFSCSVMHEALHNHYTQKSLSLSLGK

SEQ ID NO: 172 - protein, 236 aa, Artificial Sequence
  CHAIN: Amino acid sequence of FcRn-2 antibody light chain containing signal peptide
MEWSWVFLFFLSLTGVHANFMLTQPHSVSESPGKTVTISCTGSSGSIASNYVQWYQQRPGSSPTTVIYEDNQRASGVPDRFSGSIDSSSNSASLTISGLKTEDEADYYCQSYDSSSHNWVFGGGTKLTVLGQPKANPTVTLFPPSSEELQANKATLVCLISDFYPGAVTVAWKADGSPVKAGVETTKPSKQSNNKYAASSYLSLTPEQWKSHRSYSCQVTHEGSTVEKTVAPTECS